European Patent Specification EP 3 760 209 B1, published November 22, 2023. Title: Method of Gene Therapy Specific to Ischemic Lesion. Applicant: National University Corporation Tokyo Medical and Dental University. The sequence listing filed with the application follows.

SEQUENCE LISTING (6 sequences)

SEQ ID NO: 1 - DNA, 6983 bp, Mus musculus
caggcattcaggcagcgagagcagagcagcgtagagcagcacagctgagctcgtgaggcaggagactcagcccgaggaaatcgcagataagtttttaattaaaaagattgagcagtaaaaagaattagaactctaaacttaagctaatagagtagcttatcgaaatattacttagtcttaataatctaagaagatcttaagagataacatgaaggcttatttaaacagtttgaaaaaggaaatgaggagaaaagtatttgtactgtataatggaggctgaccagagcagtttaggagattgtaaagggaggttttgtgaagttctaaaaggttctagtttgaaggtcggccttgtagattaaaacgaaggttacctaaatagaatctaagtggcatttaaaacagtaaagttgtagagaatagtttgaaaatgaggtgtagttttaaaagattgagaaaagtaggttaagttgacggccgttataaaaatccttcgactggcgcatgtacgtttgaaggcatgagttggaaacagggaagatggaagtgttaggctagccgggcgatggtggcgcacgcctttaatcctagcacttgggaggcagaggcaggcggatttctgagttcgaggccagcctggtctacagagtgagttccaggacagccagggctacacagagaaaccctgtcttgaaaaaacaaaaaggttaggctagtatttggagaaagaagattagaaaatggaagtgaaagacgaagaagacatacaggaaggtgaagaaaaagctgttagagaagataggaaaatagaagacaaagcatctttagaagacagaaaaggtacttaaaggcacaggtagtaggaagccgaagaatagaagatagaaagaagcaagatagaaaaacaaaatggaagttaagacaactttggatgccagcattcaagataggcaaagaagataagattgaggccaaaaggttggataagatataaagtcagaaggaaattatctttaaagccataagttcaaatttctgatggagcgagcagtttagaagagtctttagacagccacatacaagattgaagctagcaatcaaagctactaggactgaagtaaaaagttaaggcagaatgcctttgaagagttagaagaatattaaaagccttaacttgtagcttaattttgcttgatgacaaaaggacttttgataacagtttcaagattgtcagcattttgcattggacttgagctgaggtgcttttaaaatcctaacgactagcattggcagctgacccaggtctacacagaagtgcattcagtgaactaggaagacaggagcggcagacaggagtcccgaagccagtttggtgaagctaggaaggactgaggagccagcagcagcagtgcatggtgaagatagcccaggaaagagtgcggttcggtggaggaagctaggaagaaggagccatacggatgtggtggtgaagctgggaaagggttccaggatggtggagcgagagcgagttggtgatgaagctagctggcggcttggcttgtcaactgcgcggaggaggcgagcaggcattgtggagaggatagatagcggctcctagaccagcatgccagtgtgcaagaaaggctgcagggagagcatgcggtgcggtaacattccttgaggtcggcaacatggtggtggttttctgtaacttggatggtaacttgtttactttgtcttaatagttatgggggagttgtaggcttctgtgtaaagagatatatctggggctgtatgtaggcctttgcgggtgttgtaggtttttctttttcagggttatgtcctcttgcatcttgtcagaagcttttgagggctgactgccaaggcccagaaagaagaatggtagatggcaagttgtctttaaccgctcagaggggaatgaatggtagagccagcacaacctcccagttttgtaagacgttgtagtttgaacagatgacctaccacaagcctcactcctgtgtaggggaggtaattgggcaaagtgcttttgggggaatgggggcaaaatatattttgagttcttttccccttaggtctgtctagaatcctaaaggcagatgactcaagggaaccagaaaaaaggaaatccactctcaggataagcagagctcgccaggtttacagtttgtaggaagtagaggatggatgctagctttcacactgagtgtggaggagctggccatggcggaattgctggtagtttactctttccccctcccttaatgagatttgtaaaatcctaaacacttttacttgaaatatttgggagtggtcttaacagggaggagtgggtgggggaaacgttttttttctaagattttccacagatgctatagttgtgttgacacactgggttagagaaggcgtgtactgctatgctgttggcacgacaccttcagggactggagctgccttttgtccttggaagagttttcccagttgccgctgaagtcagcacagtgcggctttggttcacagtcacctcaggagaacctcaggagcttggctaggccagaggttgaagttaagttttacagcaccgtgatttaaaatatttcattaaaggggaggggtaaaacttagttggctgtggccttgtgtttgggtgggtgggggtgttaggtaattgtttagtttatgatttcagataatcataccagagaacttaaatatttggaaaaacaggaaatctcagctttcaagttggcaagtaactcccaatccagtttttgcttcttttttcctttttctttttttgaggcgggcagctaaggaaggttggttcctctgccggtccctcgaaagcgtagggcttgggggttggtctggtccactgggatgatgtgatgctacagtggggactcttctgaagctgttggatgaatatagattgtagtgtgtggttctcttttgaaatttttttcaggtgacttaatgtatcttaataactactataggaacaaaggaagtggctttaatgaccctgaaggaatttcttctggtgatagcttttatattatcaagtaagagatactatctcagttttgtataagcaagtctttttcctagtgtaggagaaatgattttccttgtgactaaacaagatgtaaaggtatgctttttttcttcttgtgcattgtatacttgtgtttatttgtaacttataatttaagaattatgataattcagcctgaatgtcttttagagggtgggcttttgttgatgagggaggggaaacctttttttttctgtagacctttttcagataacaccatctgagtcataaccagcctggcagtgtgatgacgtagatgcagagggagcagctccttggtgaatgagtgataagtaaaggcagaaaaaataatgtcatgtctccatggggaatgagcatgagccagagattgttcctactgatgaaaagctgcatatgcaaaaatttaagcaaatgaaagcaaccagtataaagttatggcaatacctttaaaagttatggcttatctaccaagctttatccacaaaagtaaagaattgatgaaaaacagtgaagatcaaatgttcatctcaaaactgcttttacaaaagcagaatagaaatgaagtgaaaatgctgcattaagcctggagtaaaaagaagctgagcttgttgagatgagtgggatcgagcggctgcgaggcggtgcagtgtgccaatgtttcgtttgcctcagacaggtttctcttcataagcagaagagttgcttcattccatctcggagcaggaaacagcagactgctgttgacagataagtgtaacttggatctgcagtattgcatgttagggatagataagtgccttttttctctttttccaaaaagacctgtagagctgttgaatgtttgcagctggcccctcttaggcagttcagaattttgagtagttttcccatccagcctcttaaaaattcctaagccttgcaccgatgggctttcatgatgggatagctaataggcttttgcatcgtaaacttcaacacaaaagcctacatgattaatgcctactttaattacattgcttacaagattaaggaatctttatcttgaagaccccatgaaagggatcattatgtgctgaaaattagatgttcatattgctaaaatttaaatgtgctccaatgtacttgtgcttaaaatcattaaattatacaaattaataaaatacttcactagagaatgtatgtatttagaaggctgtctccttatttaaataaagtcttgtttgttgtctgtagttagtgtgggcaattttggggggatgttcttctctaatcttttcagaaacttgacttcgaacacttaagtggaccagatcaggatttgagccagaagaccgaaattaactttaaggcaggaaagacaaattttattctccatgcagtgatgagcatttaataattgcaggcctggcatagaggccgtctaactaaggactaagtaccttaggcaggtgggagatgatggtcagagtaaaaggtaactacatattttgtttccagaaagtcaggggtctaatttgaccatggctaaacatctagggtaagacacttttcccccacatttccaaatatgcatgttgagtttaaatgcttacgatcatctcatccactttagccttttgtcacctcacttgagccacgagtggggtcaggcatgtgggtttaaagagttttcctttgcagagcctcatttcatccttcatggagctgctcaggactttgcatataagcgcttgcctctgtcttctgttctgctagtgagtgtgtgatgtgagaccttgcagtgagtttgtttttcctggaatgtggagggagggggggatggggcttacttgttctagctttttttttacagaccacacagaatgcaggtgtcttgacttcaggtcatgtctgttctttggcaagtaatatgtgcagtactgttccaatctgctgctattagaatgcattgtgacgcgactggagtatgattaaagaaagttgtgtttccccaagtgtttggagtagtggttgttggaggaaaagccatgagtaacaggctgagtgttgaggaaatggctctctgcagctttaagtaacccgtgtttgtgattggagccgagtccctttgctgtgctgccttaggtaaatgtttttgttcatttctggtgaggggggttgggagcactgaagcctttagtctcttccagattcaacttaaaatctgacaagaaataaatcagacaagcaacattcttgaagaaattttaactggcaagtggaaatgttttgaacagttccgtggtctttagtgcattatctttgtgtaggtgttctctctcccctcccttggtcttaattcttacatgcaggaacattgacaacagcagacatctatctattcaaggggccagagaatccagacccagtaaggaaaaatagcccatttactttaaatcgataagtgaagcagacatgccattttcagtgtggggattgggaagccctagttctttcagatgtacttcagactgtagaaggagcttccagttgaattgaaattcaccagtggacaaaatgaggacaacaggtgaacgagccttttcttgtttaagattagctactggtaatctagtgttgaatcctctccagcttcatgctggagcagctagcatgtgatgtaatgttggccttggggtggaggggtgaggtgggcgctaagcctttttttaagatttttcaggtacccctcactaaaggcactgaaggcttaatgtaggacagcggagccttcctgtgtggcaagaatcaagcaagcagtattgtatcgagaccaaagtggtatcatggtcggttttgattagcagtggggactaccctaccgtaacaccttgttggaattgaagcatccaaagaaaatacttgagaggccctgggcttgttttaacatctggaaaaaaggctgtttttatagcagcggttaccagcccaaacctcaagttgtgcttgcaggggagggaaaagggggaaagcgggcaaccagtttccccagcttttccagaatcctgttacaaggtctccccacaagtgatttctctgccacatcgccaccatgggcctttggcctaatcacagacccttcacccctcaccttgatgcagccagtagctggatccttgaggtcacgttgcatatcggtttcaaggtaaccatggtgccaaggtcctgtgggttgcaccagaaaaggccatcaattttccccttgcctgtaatttaacattaaaaccatagctaagatgttttatacatagcacctatgcagagtaaacaaaccagtatgggtatagtatgtttgataccagtgctgggtgggaatgtaggaagtcggatgaaaagcaagcctttgtaggaagttgttggggtgggattgcaaaaattctctgctaagactttttcaggtggacataacagacttggccaagctagcatcttagtggaagcagattcgtcagtagggttgtaaaggtttttcttttcctgagaaaacaaccttttgttttctcaggttttgctttttggcctttccctagctttaaaaaaaaaaaagcaaaagacgctggtggctggcactcctggtttccaggacggggttcaagtccctgcggtgtctttgcttgactcttatatcatgaggccattacatttttcttggagggttctaaaggctctgggtatggtagctgatatcactggaacactccccagcctcagtgttgaactcttgataattaactgcattgtctttcaggttatgcccaattcgtcttattacctctgagtcgacacacctcctactatttattgaatactttgattttatgaaataaaaactaaatatctctca

SEQ ID NO: 2 - DNA, 8779 bp, Homo sapiens
cgcagcctgcagcccgagacttctgtaaaggactggggccccgcaactggcctctcctgccctcttaagcgcagcgccattttagcaacgcagaagcccggcgccgggaagcctcagctcgcctgaaggcaggtcccctctgacgcctccgggagcccaggtttcccagagtccttgggacgcagcgacgagttgtgctgctatcttagctgtccttataggctggccattccaggtggtggtatttagataaaaccactcaaactctgcagtttggtcttggggtttggaggaaagcttttatttttcttcctgctccggttcagaaggtctgaagctcatacctaaccaggcataacacagaatctgcaaaacaaaaacccctaaaaaagcagacccagagcagtgtaaacacttctgggtgtgtccctgactggctgcccaaggtctctgtgtcttcggagacaaagccattcgcttagttggtctactttaaaaggccacttgaactcgctttccatggcgatttgccttgtgagcactttcaggagagcctggaagctgaaaaacggtagaaaaatttccgtgcgggccgtggggggctggcggcaactggggggccgcagatcagagtgggccactggcagccaacggcccccggggctcaggcggggagcagctctgtggtgtgggattgaggcgttttccaagagtgggttttcacgtttctaagatttcccaagcagacagcccgtgctgctccgatttctcgaacaaaaaagcaaaacgtgtggctgtcttgggagcaagtcgcaggactgcaagcagttgggggagaaagtccgccattttgccacttctcaaccgtccctgcaaggctggggctcagttgcgtaatggaaagtaaagccctgaactatcacactttaatcttccttcaaaaggtggtaaactatacctactgtccctcaagagaacacaagaagtgctttaagaggtattttaaaagttccgggggttttgtgaggtgtttgatgacccgtttaaaatatgatttccatgtttcttttgtctaaagtttgcagctcaaatctttccacacgctagtaatttaagtatttctgcatgtgtagtttgcattcaagttccataagctgttaagaaaaatctagaaaagtaaaactagaacctatttttaaccgaagaactactttttgcctccctcacaaaggcggcggaaggtgatcgaattccggtgatgcgagttgttctccgtctataaatacgcctcgcccgagctgtgcggtaggcattgaggcagccagcgcaggggcttctgctgagggggcaggcggagcttgaggaaaccgcagataagtttttttctctttgaaagatagagattaatacaactacttaaaaaatatagtcaataggttactaagatattgcttagcgttaagtttttaacgtaattttaatagcttaagattttaagagaaaatatgaagacttagaagagtagcatgaggaaggaaaagataaaaggtttctaaaacatgacggaggttgagatgaagcttcttcatggagtaaaaaatgtatttaaaagaaaattgagagaaaggactacagagccccgaattaataccaatagaagggcaatgcttttagattaaaatgaaggtgacttaaacagcttaaagtttagtttaaaagttgtaggtgattaaaataatttgaaggcgatcttttaaaaagagattaaaccgaaggtgattaaaagaccttgaaatccatgacgcagggagaattgcgtcatttaaagcctagttaacgcatttactaaacgcagacgaaaatggaaagattaattgggagtggtaggatgaaacaatttggagaagatagaagtttgaagtggaaaactggaagacagaagtacgggaaggcgaagaaaagaatagagaagatagggaaattagaagataaaaacatacttttagaagaaaaaagataaatttaaacctgaaaagtaggaagcagaagaaaaaagacaagctaggaaacaaaaagctaagggcaaaatgtacaaacttagaagaaaattggaagatagaaacaagatagaaaatgaaaatattgtcaagagtttcagatagaaaatgaaaaacaagctaagacaagtattggagaagtatagaagatagaaaaatataaagccaaaaattggataaaatagcactgaaaaaatgaggaaattattggtaaccaatttattttaaaagcccatcaatttaatttctggtggtgcagaagttagaaggtaaagcttgagaagatgagggtgtttacgtagaccagaaccaatttagaagaatacttgaagctagaaggggaagttggttaaaaatcacatcaaaaagctactaaaaggactggtgtaatttaaaaaaaactaaggcagaaggcttttggaagagttagaagaatttggaaggccttaaatatagtagcttagtttgaaaaatgtgaaggactttcgtaacggaagtaattcaagatcaagagtaattaccaacttaatgtttttgcattggactttgagttaagattattttttaaatcctgaggactagcattaattgacagctgacccaggtgctacacagaagtggattcagtgaatctaggaagacagcagcagacaggattccaggaaccagtgtttgatgaagctaggactgaggagcaagcgagcaagcagcagttcgtggtgaagataggaaaagagtccaggagccagtgcgatttggtgaaggaagctaggaagaaggaaggagcgctaacgatttggtggtgaagctaggaaaaaggattccaggaaggagcgagtgcaatttggtgatgaaggtagcaggcggcttggcttggcaaccacacggaggaggcgagcaggcgttgtgcgtagaggatcctagaccagcatgccagtgtgccaaggccacagggaaagcgagtggttggtaaaaatccgtgaggtcggcaatatgttgtttttctggaacttacttatggtaaccttttatttattttctaatataatgggggagtttcgtactgaggtgtaaagggatttatatggggacgtaggccgatttccgggtgttgtaggtttctctttttcaggcttatactcatgaatcttgtctgaagcttttgagggcagactgccaagtcctggagaaatagtagatggcaagtttgtgggttttttttttttacacgaatttgaggaaaaccaaatgaatttgatagccaaattgagacaatttcagcaaatctgtaagcagtttgtatgtttagttggggtaatgaagtatttcagttttgtgaatagatgacctgtttttacttcctcaccctgaattcgttttgtaaatgtagagtttggatgtgtaactgaggcgggggggagttttcagtatttttttttgtgggggtgggggcaaaatatgttttcagttctttttcccttaggtctgtctagaatcctaaaggcaaatgactcaaggtgtaacagaaaacaagaaaatccaatatcaggataatcagaccaccacaggtttacagtttatagaaactagagcagttctcacgttgaggtctgtggaagagatgtccattggagaaatggctggtagttactcttttttccccccacccccttaatcagactttaaaagtgcttaaccccttaaacttgttattttttacttgaagcattttgggatggtcttaacagggaagagagagggtgggggagaaaatgtttttttctaagattttccacagatgctatagtactattgacaaactgggttagagaaggagtgtaccgctgtgctgttggcacgaacaccttcagggactggagctgcttttatccttggaagagtattcccagttgaagctgaaaagtacagcacagtgcagctttggttcatattcagtcatctcaggagaacttcagaagagcttgagtaggccaaatgttgaagttaagttttccaataatgtgacttcttaaaagttttattaaaggggaggggcaaatattggcaattagttggcagtggcctgttacggttgggattggtggggtgggtttaggtaattgtttagtttatgattgcagataaactcatgccagagaacttaaagtcttagaatggaaaaagtaaagaaatatcaacttccaagttggcaagtaactcccaatgatttagtttttttccccccagtttgaattgggaagctgggggaagttaaatatgagccactgggtgtaccagtgcattaatttgggcaaggaaagtgtcataatttgatactgtatctgttttccttcaaagtatagagcttttggggaaggaaagtattgaactgggggttggtctggcctactgggctgacattaactacaattatgggaaatgcaaaagttgtttggatatggtagtgtgtggttctcttttggaatttttttcaggtgatttaataataatttaaaactactatagaaactgcagagcaaaggaagtggcttaatgatcctgaagggatttcttctgatggtagcttttgtattatcaagtaagattctattttcagttgtgtgtaagcaagtttttttttagtgtaggagaaatacttttccattgtttaactgcaaaacaagatgttaaggtatgcttcaaaaattttgtaaattgtttattttaaacttatctgtttgtaaattgtaactgattaagaattgtgatagttcagcttgaatgtctcttagagggtgggcttttgttgatgagggaggggaaactttttttttttctatagacttttttcagataacatcttctgagtcataaccagcctggcagtatgatggcctagatgcagagaaaacagctccttggtgaattgataagtaaaggcagaaaagattatatgtcatacctccattggggaataagcataaccctgagattcttactactgatgagaacattatctgcatatgccaaaaaattttaagcaaatgaaagctaccaatttaaagttacggaatctaccattttaaagttaattgcttgtcaagctataaccacaaaaataatgaattgatgagaaatacaatgaagaggcaatgtccatctcaaaatactgcttttacaaaagcagaataaaagcgaaaagaaatgaaaatgttacactacattaatcctggaataaaagaagccgaaataaatgagagatgagttgggatcaagtggattgaggaggctgtgctgtgtgccaatgtttcgtttgcctcagacaggtatctcttcgttatcagaagagttgcttcatttcatctgggagcagaaaacagcaggcagctgttaacagataagtttaacttgcatctgcagtattgcatgttagggataagtgcttatttttaagagctgtggagttcttaaatatcaaccatggcactttctcctgaccccttccctaggggatttcaggattgagaaatttttccatcgagcctttttaaaattgtaggacttgttcctgtgggcttcagtgatgggatagtacacttcactcagaggcatttgcatctttaaataatttcttaaaagcctctaaagtgatcagtgccttgatgccaactaaggaaatttgtttagcattgaatctctgaaggctctatgaaaggaatagcatgatgtgctgttagaatcagatgttactgctaaaatttacatgttgtgatgtaaattgtgtagaaaaccattaaatcattcaaaataataaactatttttattagagaatgtatacttttagaaagctgtctccttatttaaataaaatagtgtttgtctgtagttcagtgttggggcaatcttgggggggattcttctctaatctttcagaaactttgtctgcgaacactctttaatggaccagatcaggatttgagcggaagaacgaatgtaactttaaggcaggaaagacaaattttattcttcataaagtgatgagcatataataattccaggcacatggcaatagaggccctctaaataaggaataaataacctcttagacaggtgggagattatgatcagagtaaaaggtaattacacattttatttccagaaagtcaggggtctataaattgacagtgattagagtaatactttttcacatttccaaagtttgcatgttaactttaaatgcttacaatcttagagtggtaggcaatgttttacactattgaccttatatagggaagggagggggtgcctgtggggttttaaagaattttcctttgcagaggcatttcatccttcatgaagccattcaggattttgaattgcatatgagtgcttggctcttccttctgttctagtgagtgtatgagaccttgcagtgagtttatcagcatactcaaaatttttttcctggaatttggagggatgggaggagggggtggggcttacttgttgtagctttttttttttttacagacttcacagagaatgcagttgtcttgacttcaggtctgtctgttctgttggcaagtaaatgcagtactgttctgatcccgctgctattagaatgcattgtgaaacgactggagtatgattaaaagttgtgttccccaatgcttggagtagtgattgttgaaggaaaaaatccagctgagtgataaaggctgagtgttgaggaaatttctgcagttttaagcagtcgtatttgtgattgaagctgagtacattttgctggtgtatttttaggtaaaatgctttttgttcatttctggtggtgggaggggactgaagcctttagtcttttccagatgcaaccttaaaatcagtgacaagaaacattccaaacaagcaacagtcttcaagaaattaaactggcaagtggaaatgtttaaacagttcagtgatctttagtgcattgtttatgtgtgggtttctctctcccctcccttggtcttaattcttacatgcaggaacactcagcagacacacgtatgcgaagggccagagaagccagacccagtaagaaaaaatagcctatttactttaaataaaccaaacattccattttaaatgtggggattgggaaccactagttctttcagatggtattcttcagactatagaaggagcttccagttgaattcaccagtggacaaaatgaggaaaacaggtgaacaagctttttctgtatttacatacaaagtcagatcagttatgggacaatagtattgaatagatttcagctttatgctggagtaactggcatgtgagcaaactgtgttggcgtgggggtggaggggtgaggtgggcgctaagcctttttttaagatttttcaggtacccctcactaaaggcaccgaaggcttaaagtaggacaaccatggagccttcctgtggcaggagagacaacaaagcgctattatcctaaggtcaagagaagtgtcagcctcacctgatttttattagtaatgaggacttgcctcaactccctctttctggagtgaagcatccgaaggaatgcttgaagtacccctgggcttctcttaacatttaagcaagctgtttttatagcagctcttaataataaagcccaaatctcaagcggtgcttgaaggggagggaaagggggaaagcgggcaaccacttttccctagcttttccagaagcctgttaaaagcaaggtctccccacaagcaacttctctgccacatcgccaccccgtgccttttgatctagcacagacccttcacccctcacctcgatgcagccagtagcttggatccttgtgggcatgatccataatcggtttcaaggtaacgatggtgtcgaggtctttggtgggttgaactatgttagaaaaggccattaatttgcctgcaaattgttaacagaagggtattaaaaccacagctaagtagctctattataatacttatccagtgactaaaaccaacttaaaccagtaagtggagaaataacatgttcaagaactgtaatgctgggtgggaacatgtaacttgtagactggagaagataggcatttgagtggctgagagggcttttgggtgggaatgcaaaaattctctgctaagactttttcaggtgaacataacagacttggccaagctagcatcttagcggaagctgatctccaatgctcttcagtagggtcatgaaggtttttcttttcctgagaaaacaacacgtattgttttctcaggttttgctttttggcctttttctagcttaaaaaaaaaaaaagcaaaagatgctggtggttggcactcctggtttccaggacggggttcaaatccctgcggcgtctttgctttgactactaatctgtcttcaggactctttctgtatttctccttttctctgcaggtgctagttcttggagttttggggaggtgggaggtaacagcacaatatctttgaactatatacatccttgatgtataatttgtcaggagcttgacttgattgtatattcatatttacacgagaacctaatataactgccttgtctttttcaggtaatagcctgcagctggtgttttgagaagccctactgctgaaaacttaacaattttgtgtaataaaaatggagaagctctaaattgttgtggttcttttgtgaataaaaaaatcttgattggggaaaaaa

SEQ ID NO: 3 - DNA, 16 bp, Artificial
  Synthetic
  misc_feature (1)..(3): LNA
  misc_feature (14)..(16): LNA
ctagttcactgaatgc

SEQ ID NO: 4 - RNA, 16 nt, Artificial
  Synthetic
  misc_feature (1)..(3): 2'-O-Me RNA
  misc_feature (14)..(16): 2'-O-Me RNA
gcauucagugaacuag

SEQ ID NO: 5 - DNA, 16 bp, Artificial
  Synthetic
  misc_feature (1)..(3): LNA
  misc_feature (14)..(16): LNA
tacatatgcgctactg

SEQ ID NO: 6 - RNA, 16 nt, Artificial
  Synthetic
  misc_feature (1)..(3): 2'-O-Me RNA
  misc_feature (14)..(16): 2'-O-Me RNA
caguagcgcauaugua